European Patent Application EP 4 781 997 A1, published July 29, 2026. Title: LACTICASEIBACILLUS STRAIN AND USES THEREOF. Applicant: KERRY GROUP SERVICES INTERNATIONAL LIMITED. Application EP. The sequence listing filed with the application follows.

SEQUENCE LISTING (5 sequences)

SEQ ID NO: 1 - DNA, 1551 bp, unidentified
  source 1..1551: mol_type = unassigned DNA
agagtttgatcctggctcaggatgaacgctggcggcgtgcctaatacatgcaagtcgaacgagttctcgttgatgatcggtgcttgcaccgagattcaacatggaacgagtggcggacgggtgagtaacacgtgggtaacctgcccttaagtgggggataacatttggaaacagatgctaataccgcatagatccaagaaccgcatggttcttggctgaaagatggcgtaagctatcgcttttggatggacccgcggcgtattagctagttggtgaggtaatggctcaccaaggcgatgatacgtagccgaactgagaggttgatcggccacattgggactgagacacggcccaaactcctacgggaggcagcagtagggaatcttccacaatggacgcaagtctgatggagcaacgccgcgtgagtgaagaaggctttcgggtcgtaaaactctgttgttggagaagaatggtcggcagagtaactgttgtcggcgtgacggtatccaaccagaaagccacggctaactacgtgccagcagccgcggtaatacgtaggtggcaagcgttatccggatttattgggcgtaaagcgagcgcaggcggttttttaagtctgatgtgaaagccctcggcttaaccgaggaagcgcatcggaaactgggaaacttgagtgcagaagaggacagtggaactccatgtgtagcggtgaaatgcgtagatatatggaagaacaccagtggcgaaggcggctgtctggtctgtaactgacgctgaggctcgaaagcatgggtagcgaacaggattagataccctggtagtccatgccgtaaacgatgaatgctaggtgttggagggtttccgcccttcagtgccgcagctaacgcattaagcattccgcctggggagtacgaccgcaaggttgaaactcaaaggaattgacgggggcccgcacaagcggtggagcatgtggtttaattcgaagcaacgcgaagaaccttaccaggtcttgacatcttttgatcacctgagagatcaggtttccccttcgggggcaaaatgacaggtggtgcatggttgtcgtcagctcgtgtcgtgagatgttgggttaagtcccgcaacgagcgcaacccttatgactagttgccagcatttagttgggcactctagtaagactgccggtgacaaaccggaggaaggtggggatgacgtcaaatcatcatgccccttatgacctgggctacacacgtgctacaatggatggtacaacgagttgcgagaccgcgaggtcaagctaatctcttaaagccattctcagttcggactgtaggctgcaactcgcctacacgaagtcggaatcgctagtaatcgcggatcagcacgccgcggtgaatacgttcccgggccttgtacacaccgcccgtcacaccatgagagtttgtaacacccgaagccggtggcgtaacccttttagggagcgagccgtctaaggtgggacaaatgattagggtgaagtcgtaacaaggtagccgtaggagaacctgcggctgg

SEQ ID NO: 2 - DNA, 18 bp, synthetic construct
  source 1..18: mol_type = other DNA
gctggatcacctcctttc

SEQ ID NO: 3 - DNA, 19 bp, synthetic construct
  source 1..19: mol_type = other DNA
cgatgcgaatttctttttc

SEQ ID NO: 4 - DNA, 24 bp, synthetic construct
  source 1..24: mol_type = other DNA
cccactgctgcctcccgtaggagt

SEQ ID NO: 5 - DNA, 18 bp, synthetic construct
  source 1..18: mol_type = other DNA
caccgagattcaacatgg